European Patent Application EP 4 545 554 A1, published April 30, 2025. Title: A RECOMBINANT POLYPEPTIDE COMPRISING A METAL-BINDING MOTIF. Applicant: Hober Biotech. Application EP. The sequence listing filed with the application follows.

SEQUENCE LISTING (39 sequences)

SEQ ID NO: 1-2 - skipped (2 entries)

SEQ ID NO: 3 - protein, 65 aa, synthetic construct
TTYKLILNGKTLKGETTTEXXXXXXXXXXXXXXXXEKVFKQYANDNGVDGEWTYDDATKTFTVTE

SEQ ID NO: 4 - protein, 65 aa, synthetic construct
TTYKLVINGKTLKGETTTEXXXXXXXXXXXXXXXXEKVFKQYANDNGVDGEWTYDDATKTFTVTE

SEQ ID NO: 5 - protein, 65 aa, synthetic construct
TTYKLVINGKTLKGETTTKXXXXXXXXXXXXXXXXEKAFKQYANDNGVDGVWTYDDATKTFTVTE

SEQ ID NO: 6 - protein, 13 aa, synthetic construct
DVNNDGFIDFEDA

SEQ ID NO: 7 - protein, 13 aa, synthetic construct
DKDGDGRLNYKDA

SEQ ID NO: 8 - protein, 13 aa, synthetic construct
DVNRDGKINAKDA

SEQ ID NO: 9 - protein, 13 aa, synthetic construct
DTNKDGFVDFKDA

SEQ ID NO: 10 - protein, 13 aa, synthetic construct
DVNKDGRVDFKDA

SEQ ID NO: 11 - protein, 13 aa, synthetic construct
DTNNDGYVNFKDA

SEQ ID NO: 12 - protein, 13 aa, synthetic construct
DTNRDGRVDYKDA

SEQ ID NO: 13 - protein, 13 aa, synthetic construct
DTNRDGKVTFEDA

SEQ ID NO: 14 - protein, 13 aa, synthetic construct
DKNNDGKINYKDA

SEQ ID NO: 15 - protein, 13 aa, synthetic construct
DANRDGRIDAKDA

SEQ ID NO: 16 - protein, 13 aa, synthetic construct
DEDGNGYINFEDA

SEQ ID NO: 17 - protein, 13 aa, synthetic construct
DANKDGKINAKDA

SEQ ID NO: 18 - protein, 13 aa, synthetic construct
DANRDGRINADDA

SEQ ID NO: 19 - protein, 13 aa, synthetic construct
DANKDGKINAEDA

SEQ ID NO: 20 - protein, 64 aa, synthetic construct
TTYKLVINGKTLKGETTTEPPDVNNDGFIDFEDAGKVFKQYANDNGVDGEWTYDDATKTFTVTE

SEQ ID NO: 21 - protein, 64 aa, synthetic construct
TTYKLVINGKTLKGETTTEPPDVNNDGRIDFEDAGKVFKQYANDNGVDGEWTYDDATKTFTVTE

SEQ ID NO: 22 - protein, 64 aa, synthetic construct
TTYKLVINGKTLKGETTTEPPDVNNDGYIDFEDAGKVFKQYANDNGVDGEWTYDDATKTFTVTE

SEQ ID NO: 23 - protein, 64 aa, synthetic construct
TTYKLVINGKTLKGETTTEPPDVNNDGHIDFEDAGKVFKQYANDNGVDGEWTYDDATKTFTVTE

SEQ ID NO: 24 - protein, 64 aa, synthetic construct
TTYKLVINGKTLKGETTTEPPDVNKDGFIDFEDAGKVFKQYANDNGVDGEWTYDDATKTFTVTE

SEQ ID NO: 25 - protein, 64 aa, synthetic construct
TTYKLILNGKTLKGETTTEPPDVNNDGFIDFEDAGKVFKQYANDNGVDGEWTYDDATKTFTVTE

SEQ ID NO: 26 - protein, 65 aa, synthetic construct
TTYKLVINGKTLKGETTTEPTSDKDGDGRLNYKDAEKVFKQYANDNGVDGEWTYDDATKTFTVTE

SEQ ID NO: 27 - protein, 64 aa, synthetic construct
TTYKLVINGKTLKGETTTEPPDVNRDGKINAKDAEKVFKQYADDNGVDGEWTYDDATKTFTVTE

SEQ ID NO: 28 - protein, 64 aa, synthetic construct
TTYKLVINGKTLKGETTTDPSDTNKDGFVDFKDAEKVFKQYANDNGVDGEWTYDDATKTFTVTE

SEQ ID NO: 29 - protein, 64 aa, synthetic construct
TTYKLVINGKTLKGETTTEPPDVNKDGRVDFKDAEKVFKQYANDNGVDGEWTYDDATKTFTVTE

SEQ ID NO: 30 - protein, 64 aa, synthetic construct
TTYKLVINGKTLKGETTTEPGDTNNDGYVNFKDAEKVFKQYANDNGVDGEWTYDDATKTFTVTE

SEQ ID NO: 31 - protein, 64 aa, synthetic construct
TTYKLVINGKTLKGETTTEPPDTNRDGRVDYKDAEKVFKQYANDNGVDGEWTYDDATKTFTVTE

SEQ ID NO: 32 - protein, 64 aa, synthetic construct
TTYKLVINGKTLKGETTTEPGDTNRDGKVTFEDAEKVFKQYANDNGVDGEWTYDDATKTFTVTE

SEQ ID NO: 33 - protein, 65 aa, synthetic construct
TTYKLVINGKTLKGETTTETGTDKNNDGKINYKDAEKVFKQYANDNGVDGEWTYDDATKTFTVTE

SEQ ID NO: 34 - protein, 64 aa, synthetic construct
TTYKLVINGKTLKGETTTEPPDANRDGRIDAKDAEKVFKQYANDNGVDGEWTYDDATKTFTVTE

SEQ ID NO: 35 - protein, 64 aa, synthetic construct
TTYKLVINGKTLKGETTTEPGDENGNGYINFEDAEKVFKQYANDNGVDGEWTYDDATKTFTVTE

SEQ ID NO: 36 - protein, 64 aa, synthetic construct
TTYKLVINGKTLKGETTTEPGDANKDGKINAKDAEKVFKQYANDNGVDGEWTYDDATKTFTVTE

SEQ ID NO: 37 - protein, 64 aa, synthetic construct
TTYKLVINGKTLKGETTTEPSDANRDGRINADDAEKVFKQYANDNGVDGEWTYDDATKTFTVTE

SEQ ID NO: 38 - protein, 64 aa, synthetic construct
TTYKLVINGKTLKGETTTEPGDANKDGKINAEDAEKVFKQYANDNGVDGEWTYDDATKTFTVTE

SEQ ID NO: 39 - DNA, 192 bp, synthetic construct
  source 1..192: mol_type = other DNA
accacttacaaacttgttattaatggtaaaacattgaaaggcgaaacaactacagaaccaccagatgtaaataacgatggctttatagactttgaggacgcgggaaaagtcttcaaacaatacgctaacgacaacggtgttgacggtgaatggacttacgacgatgcgactaagacctttacagttactgaa